European Patent Application EP 4 282 884 A1, published November 29, 2023. Title: MULTI-DOMAIN FUSION PROTEIN AND USE THEREOF. Applicant: ZHEJIANG DOER BIOLOGICS CO., LTD. The sequence listing filed with the application follows.

SEQUENCE LISTING (56 sequences)

SEQ ID NO: 1 - protein, 8 aa, Artificial Sequence
GSIFSANL

SEQ ID NO: 2 - protein, 8 aa, Artificial Sequence
GGTFITYA

SEQ ID NO: 3 - protein, 8 aa, Artificial Sequence
GRAFLTYA

SEQ ID NO: 4 - protein, 8 aa, Artificial Sequence
GRPFITYA

SEQ ID NO: 5 - protein, 8 aa, Artificial Sequence
GRTFSTHS

SEQ ID NO: 6 - protein, 7 aa, Artificial Sequence
ISSRGIT

SEQ ID NO: 7 - protein, 8 aa, Artificial Sequence
ISWSGSST

SEQ ID NO: 8 - protein, 8 aa, Artificial Sequence
INWSGSIT

SEQ ID NO: 9 - protein, 8 aa, Artificial Sequence
INWNGDST

SEQ ID NO: 10 - protein, 10 aa, Artificial Sequence
HLFHTDGLGY

SEQ ID NO: 11 - protein, 18 aa, Artificial Sequence
AAKISGATREHLMTSYDY

SEQ ID NO: 12 - protein, 18 aa, Artificial Sequence
AAKVSGATRDHLMTTYDY

SEQ ID NO: 13 - protein, 17 aa, Artificial Sequence
ASKRTAVAPRALNDYDF

SEQ ID NO: 14 - protein, 18 aa, Artificial Sequence
AAKISGATREHLRTSYDY

SEQ ID NO: 15 - protein, 16 aa, Artificial Sequence
AARPGAPSTIVAMLDY

SEQ ID NO: 16 - protein, 116 aa, Artificial Sequence
QVQLVESGGGLVQPGGSLRLSCAASGSIFSANLIDWYRQAPGKGLELVAVISSRGITSYADSVKGRFTISRDNSKNTLYLQMNSLRAEDTAVYYCHLFHTDGLGYWGQGTLVTVSS

SEQ ID NO: 17 - protein, 125 aa, Artificial Sequence
QVQLVESGGGLVQPGGSLRLSCAASGGTFITYAMGWFRQAPGKGLEFVAGISWSGSSTYYADSVKGRFTISRDNSKNTLYLQMNSLRAEDTAVYYCAAKISGATREHLMTSYDYWGQGTLVTVSS

SEQ ID NO: 18 - protein, 125 aa, Artificial Sequence
QVQLVESGGGLVQPGGSLRLSCAASGRAFLTYAMGWFRQAPGKGLEFVAAISWSGSSTYYADSVKGRFTISRDNSKNTLYLQMNSLRAEDTAVYYCAAKVSGATRDHLMTTYDYWGQGTLVTVSS

SEQ ID NO: 19 - protein, 124 aa, Artificial Sequence
QVQLVESGGGLVQPGGSLRLSCAASGRPFITYAMGWFRQAPGKGLEFVAAINWSGSITAYADSVKGRFTISRDNSKNTLYLQMNSLRAEDTAVYYCASKRTAVAPRALNDYDFWGQGTLVTVSS

SEQ ID NO: 20 - protein, 125 aa, Artificial Sequence
QVQLVESGGGLVQPGGSLRLSCAASGGTFITYAMGWFRQAPGKGLEFVAGISWSGSSTYYADSVKGRFTISRDNSKNTLYLQMNSLRAEDTAVYYCAAKISGATREHLRTSYDYWGQGTLVTVSS

SEQ ID NO: 21 - protein, 123 aa, Artificial Sequence
QVQLVESGGGLVQPGGSLRLSCAASGRTFSTHSMGWFRQAPGKGLEFVAAINWNGDSTYYADSVKGRFTISRDNSKNTLYLQMNSLRAEDTAVYYCAARPGAPSTIVAMLDYWGQGTLVTVSS

SEQ ID NO: 22 - protein, 453 aa, Artificial Sequence
EVQLVESGGGLVQPGGSLRLSCAASGYTFTNYGMNWVRQAPGKGLEWVGWINTYTGEPTYAADFKRRFTFSLDTSKSTAYLQMNSLRAEDTAVYYCAKYPHYYGSSHWYFDVWGQGTLVTVSSASTKGPSVFPLAPSSKSTSGGTAALGCLVKDYFPEPVTVSWNSGALTSGVHTFPAVLQSSGLYSLSSVVTVPSSSLGTQTYICNVNHKPSNTKVDKKVEPKSCDKTHTCPPCPAPELLGGPSVFLFPPKPKDTLMISRTPEVTCVVVDVSHEDPEVKFNWYVDGVEVHNAKTKPREEQYNSTYRVVSVLTVLHQDWLNGKEYKCKVSNKALPAPIEKTISKAKGQPREPQVYTLPPSREEMTKNQVSLTCLVKGFYPSDIAVEWESNGQPENNYKTTPPVLDSDGSFFLYSKLTVDKSRWQQGNVFSCSVMHEALHNHYTQKSLSLSPGK

SEQ ID NO: 23 - protein, 214 aa, Artificial Sequence
DIQMTQSPSSLSASVGDRVTITCSASQDISNYLNWYQQKPGKAPKVLIYFTSSLHSGVPSRFSGSGSGTDFTLTISSLQPEDFATYYCQQYSTVPWTFGQGTKVEIKRTVAAPSVFIFPPSDEQLKSGTASVVCLLNNFYPREAKVQWKVDNALQSGNSQESVTEQDSKDSTYSLSSTLTLSKADYEKHKVYACEVTHQGLSSPVTKSFNRGEC

SEQ ID NO: 24 - protein, 136 aa, Artificial Sequence
IPPHVQKSVNNDMIVTDNNGAVKFPQLCKFCDVRFSTCDNQKSCMSNCSITSICEKPQEVCVAVWRKNDENITLETVCHDPKLPYHDFILEDAASPKCIMKEKKKPGETFFMCSCSSDECNDNIIFSEEYNTSNPD

SEQ ID NO: 25 - protein, 610 aa, Artificial Sequence
EVQLVESGGGLVQPGGSLRLSCAASGYTFTNYGMNWVRQAPGKGLEWVGWINTYTGEPTYAADFKRRFTFSLDTSKSTAYLQMNSLRAEDTAVYYCAKYPHYYGSSHWYFDVWGQGTLVTVSSASTKGPSVFPLAPSSKSTSGGTAALGCLVKDYFPEPVTVSWNSGALTSGVHTFPAVLQSSGLYSLSSVVTVPSSSLGTQTYICNVNHKPSNTKVDKKVEPKSCDKTHTCPPCPAPELLGGPSVFLFPPKPKDTLYITREPEVTCVVVDVSHEDPEVKFNWYVDGVEVHNAKTKPREEQYNSTYRVVSVLTVLHQDWLNGKEYKCKVSNKALPAPIEKTISKAKGQPREPQVYTLPPSREEMTKNQVSLTCLVKGFYPSDIAVEWESNGQPENNYKTTPPVLDSDGSFFLYSKLTVDKSRWQQGNVFSCSVMHEALHNHYTQKSLSLSPGAGGGGSGGGGSGGGGSGGGGSGIPPHVQKSVNNDMIVTDNNGAVKFPQLCKFCDVRFSTCDNQKSCMSNCSITSICEKPQEVCVAVWRKNDENITLETVCHDPKLPYHDFILEDAASPKCIMKEKKKPGETFFMCSCSSDECNDNIIFSEEYNTSNPD

SEQ ID NO: 26 - protein, 330 aa, Artificial Sequence
QVQLVESGGGLVQPGGSLRLSCAASGSIFSANLIDWYRQAPGKGLELVAVISSRGITSYADSVKGRFTISRDNSKNTLYLQMNSLRAEDTAVYYCHLFHTDGLGYWGQGTLVTVSSDIQMTQSPSSLSASVGDRVTITCSASQDISNYLNWYQQKPGKAPKVLIYFTSSLHSGVPSRFSGSGSGTDFTLTISSLQPEDFATYYCQQYSTVPWTFGQGTKVEIKRTVAAPSVFIFPPSDEQLKSGTASVVCLLNNFYPREAKVQWKVDNALQSGNSQESVTEQDSKDSTYSLSSTLTLSKADYEKHKVYACEVTHQGLSSPVTKSFNRGEC

SEQ ID NO: 27 - protein, 339 aa, Artificial Sequence
QVQLVESGGGLVQPGGSLRLSCAASGGTFITYAMGWFRQAPGKGLEFVAGISWSGSSTYYADSVKGRFTISRDNSKNTLYLQMNSLRAEDTAVYYCAAKISGATREHLRTSYDYWGQGTLVTVSSDIQMTQSPSSLSASVGDRVTITCSASQDISNYLNWYQQKPGKAPKVLIYFTSSLHSGVPSRFSGSGSGTDFTLTISSLQPEDFATYYCQQYSTVPWTFGQGTKVEIKRTVAAPSVFIFPPSDEQLKSGTASVVCLLNNFYPREAKVQWKVDNALQSGNSQESVTEQDSKDSTYSLSSTLTLSKADYEKHKVYACEVTHQGLSSPVTKSFNRGEC

SEQ ID NO: 28 - protein, 338 aa, Artificial Sequence
QVQLVESGGGLVQPGGSLRLSCAASGRPFITYAMGWFRQAPGKGLEFVAAINWSGSITAYADSVKGRFTISRDNSKNTLYLQMNSLRAEDTAVYYCASKRTAVAPRALNDYDFWGQGTLVTVSSDIQMTQSPSSLSASVGDRVTITCSASQDISNYLNWYQQKPGKAPKVLIYFTSSLHSGVPSRFSGSGSGTDFTLTISSLQPEDFATYYCQQYSTVPWTFGQGTKVEIKRTVAAPSVFIFPPSDEQLKSGTASVVCLLNNFYPREAKVQWKVDNALQSGNSQESVTEQDSKDSTYSLSSTLTLSKADYEKHKVYACEVTHQGLSSPVTKSFNRGEC

SEQ ID NO: 29 - protein, 337 aa, Artificial Sequence
QVQLVESGGGLVQPGGSLRLSCAASGRTFSTHSMGWFRQAPGKGLEFVAAINWNGDSTYYADSVKGRFTISRDNSKNTLYLQMNSLRAEDTAVYYCAARPGAPSTIVAMLDYWGQGTLVTVSSDIQMTQSPSSLSASVGDRVTITCSASQDISNYLNWYQQKPGKAPKVLIYFTSSLHSGVPSRFSGSGSGTDFTLTISSLQPEDFATYYCQQYSTVPWTFGQGTKVEIKRTVAAPSVFIFPPSDEQLKSGTASVVCLLNNFYPREAKVQWKVDNALQSGNSQESVTEQDSKDSTYSLSSTLTLSKADYEKHKVYACEVTHQGLSSPVTKSFNRGEC

SEQ ID NO: 30 - protein, 610 aa, Artificial Sequence
EVQLVESGGGLVQPGGSLRLSCAASGYTFTNYGMNWVRQAPGKGLEWVGWINTYTGEPTYAADFKRRFTFSLDTSKSTAYLQMNSLRAEDTAVYYCAKYPHYYGSSHWYFDVWGQGTLVTVSSASTKGPSVFPLAPSSKSTSGGTAALGCLVKDYFPEPVTVSWNSGALTSGVHTFPAVLQSSGLYSLSSVVTVPSSSLGTQTYICNVNHKPSNTKVDKKVEPKSCDKTHTCPPCPAPELLGGPSVFLFPPKPKDTLMISRTPEVTCVVVDVSHEDPEVKFNWYVDGVEVHNAKTKPREEQYNSTYRVVSVLTVLHQDWLNGKEYKCKVSNKALPAPIEKTISKAKGQPREPQVYTLPPSREEMTKNQVSLTCLVKGFYPSDIAVEWESNGQPENNYKTTPPVLDSDGSFFLYSKLTVDKSRWQQGNVFSCSVMHEALHNHYTQKSLSLSPGAGGGGSGGGGSGGGGSGGGGSGIPPHVQKSVNNDMIVTDNNGAVKFPQLCKFCDVRFSTCDNQKSCMSNCSITSICEKPQEVCVAVWRKNDENITLETVCHDPKLPYHDFILEDAASPKCIMKEKKKPGETFFMCSCSSDECNDNIIFSEEYNTSNPD

SEQ ID NO: 31 - protein, 735 aa, Artificial Sequence
QVQLVESGGGLVQPGGSLRLSCAASGGTFITYAMGWFRQAPGKGLEFVAGISWSGSSTYYADSVKGRFTISRDNSKNTLYLQMNSLRAEDTAVYYCAAKISGATREHLRTSYDYWGQGTLVTVSSEVQLVESGGGLVQPGGSLRLSCAASGYTFTNYGMNWVRQAPGKGLEWVGWINTYTGEPTYAADFKRRFTFSLDTSKSTAYLQMNSLRAEDTAVYYCAKYPHYYGSSHWYFDVWGQGTLVTVSSASTKGPSVFPLAPSSKSTSGGTAALGCLVKDYFPEPVTVSWNSGALTSGVHTFPAVLQSSGLYSLSSVVTVPSSSLGTQTYICNVNHKPSNTKVDKKVEPKSCDKTHTCPPCPAPELLGGPSVFLFPPKPKDTLMISRTPEVTCVVVDVSHEDPEVKFNWYVDGVEVHNAKTKPREEQYNSTYRVVSVLTVLHQDWLNGKEYKCKVSNKALPAPIEKTISKAKGQPREPQVYTLPPSREEMTKNQVSLTCLVKGFYPSDIAVEWESNGQPENNYKTTPPVLDSDGSFFLYSKLTVDKSRWQQGNVFSCSVMHEALHNHYTQKSLSLSPGAGGGGSGGGGSGGGGSGGGGSGIPPHVQKSVNNDMIVTDNNGAVKFPQLCKFCDVRFSTCDNQKSCMSNCSITSICEKPQEVCVAVWRKNDENITLETVCHDPKLPYHDFILEDAASPKCIMKEKKKPGETFFMCSCSSDECNDNIIFSEEYNTSNPD

SEQ ID NO: 32 - protein, 735 aa, Artificial Sequence
QVQLVESGGGLVQPGGSLRLSCAASGGTFITYAMGWFRQAPGKGLEFVAGISWSGSSTYYADSVKGRFTISRDNSKNTLYLQMNSLRAEDTAVYYCAAKISGATREHLRTSYDYWGQGTLVTVSSEVQLVESGGGLVQPGGSLRLSCAASGYTFTNYGMNWVRQAPGKGLEWVGWINTYTGEPTYAADFKRRFTFSLDTSKSTAYLQMNSLRAEDTAVYYCAKYPHYYGSSHWYFDVWGQGTLVTVSSASTKGPSVFPLAPSSKSTSGGTAALGCLVKDYFPEPVTVSWNSGALTSGVHTFPAVLQSSGLYSLSSVVTVPSSSLGTQTYICNVNHKPSNTKVDKKVEPKSCDKTHTCPPCPAPELLGGPSVFLFPPKPKDTLMISRTPEVTCVVVDVSHEDPEVKFNWYVDGVEVHNAKTKPREEQYASTYRVVSVLTVLHQDWLNGKEYKCKVSNKALPAPIEKTISKAKGQPREPQVYTLPPSREEMTKNQVSLTCLVKGFYPSDIAVEWESNGQPENNYKTTPPVLDSDGSFFLYSKLTVDKSRWQQGNVFSCSVMHEALHNHYTQKSLSLSPGAGGGGSGGGGSGGGGSGGGGSGIPPHVQKSVNNDMIVTDNNGAVKFPQLCKFCDVRFSTCDNQKSCMSNCSITSICEKPQEVCVAVWRKNDENITLETVCHDPKLPYHDFILEDAASPKCIMKEKKKPGETFFMCSCSSDECNDNIIFSEEYNTSNPD

SEQ ID NO: 33 - protein, 735 aa, Artificial Sequence
QVQLVESGGGLVQPGGSLRLSCAASGGTFITYAMGWFRQAPGKGLEFVAGISWSGSSTYYADSVKGRFTISRDNSKNTLYLQMNSLRAEDTAVYYCAAKISGATREHLRTSYDYWGQGTLVTVSSEVQLVESGGGLVQPGGSLRLSCAASGYTFTNYGMNWVRQAPGKGLEWVGWINTYTGEPTYAADFKRRFTFSLDTSKSTAYLQMNSLRAEDTAVYYCAKYPHYYGSSHWYFDVWGQGTLVTVSSASTKGPSVFPLAPSSKSTSGGTAALGCLVKDYFPEPVTVSWNSGALTSGVHTFPAVLQSSGLYSLSSVVTVPSSSLGTQTYICNVNHKPSNTKVDKKVEPKSCDKTHTCPPCPAPELLGGPSVFLFPPKPKDTLMISRTPEVTCVVVDVSHEDPEVKFNWYVDGVEVHNAKTKPREEQYNSTYRVVSVLTVLHQDWLNGKEYKCKVSNKALPAPIEKTISKAKGQPREPQVYTLPPSREEMTKNQVSLTCLVKGFYPSDIAVEWESNGQPENNYKTTPPVLDSDGSFFLYSKLTVDKSRWQQGNVFSCSVMHEALHNHYTQKSLSLSPGAGGGGSGGGGSGGGGSGGGGSTIPPHVQKSVNNDMIVTDNNGAVKFPQLCKFCDVRFSTCDNQKSCMSNCSITSICEKPQEVCVAVWRKNDENITLETVCHDPKLPYHDFILEDAASPKCIMKEKKKPGETFFMCSCSSDECNDNIIFSEEYNTSNPD

SEQ ID NO: 34 - protein, 15 aa, Artificial Sequence
GGGGSGGGGSGGGGS

SEQ ID NO: 35 - protein, 20 aa, Artificial Sequence
GGGGSGGGGSGGGGSGGGGS

SEQ ID NO: 36 - protein, 21 aa, Artificial Sequence
GGGGSGGGGSGGGGSGGGGSG

SEQ ID NO: 37 - DNA, 1830 bp, Artificial Sequence
gaggtgcagctggtggagtctggaggaggactggtgcagccaggaggctctctgagactgtcctgcgccgctagcggctacaccttcacaaactatggcatgaattgggtgcgccaggctccaggcaagggcctggagtgggtgggctggatcaacacctacacaggcgagcccacctatgccgctgactttaagaggaggttcaccttctccctggacacctccaagagcacagcctacctccagatgaactccctgagggccgaggacaccgccgtgtactattgcgctaagtacccccactactatggctccagccattggtatttcgacgtgtggggacagggcaccctggtgacagtgtcttccgcctctaccaagggaccttccgtgtttcctctggctccaagctctaagtctacctccggaggaacagccgctctgggatgtctggtgaaggactatttccctgagccagtgaccgtgtcctggaacagcggcgccctgacctccggagtgcacacatttcctgctgtgctccagtccagcggcctgtacagcctgtcttccgtggtgaccgtgccaagctcttccctgggcacccagacatatatctgcaacgtgaatcacaagccatccaacacaaaggtggacaagaaggtggagcccaagtcctgcgacaaaactcacacatgcccaccgtgcccagcacctgaactcctgggtggaccgtcagtcttcctcttccccccaaaacccaaggacaccctctacatcacccgggaacctgaggtcacatgcgtggtggtggacgtgagccacgaagaccctgaggtcaagttcaactggtacgtggacggcgtggaggtgcataatgccaagacaaagccgcgggaggagcagtacaatagcacgtaccgtgtggtcagcgtcctcaccgtcctgcaccaggactggctgaatggcaaggagtacaagtgcaaggtctccaacaaagccctcccagcccccatcgagaaaaccatctccaaagccaaagggcagccccgagaaccacaggtgtacaccctgcccccatcccgggaggagatgaccaagaaccaggtcagcctgacctgcctggtcaaaggcttctatcccagcgacatcgccgtggagtgggagagcaatgggcagccggagaacaactacaagaccacgcctcccgtgctggactccgacggctccttcttcctctatagcaagctcaccgtggacaagagcaggtggcagcaggggaacgtcttctcatgctccgtgatgcatgaggctctgcacaaccactacacgcagaagagcctctccctgtctccgggtgctggaggaggaggaagcggaggaggaggctctggcggcggcggctcaggcggcggcggcagcggcatccccccacacgtgcagaagtccgtgaataatgacatgatcgtgaccgataacaacggcgccgtgaagtttccccagctgtgcaagttctgcgacgtgaggttctccacctgtgacaaccagaagtcctgtatgagcaactgcagcatcacctccatctgcgagaagccccaggaggtgtgtgtggccgtgtggcggaagaacgacgagaatatcaccctggagaccgtgtgtcacgaccccaagctgccctatcacgacttcatcctggaggatgctgctagccccaagtgcatcatgaaggagaagaagaagcccggcgagaccttcttcatgtgttcctgtagcagcgacgagtgcaatgataacatcatctttagcgaggagtacaacacctccaaccccgac

SEQ ID NO: 38 - DNA, 990 bp, Artificial Sequence
caggtgcagctcgtggagtctgggggaggcttggtgcagcctggggggtctctgagactctcctgtgcagcctctggaagcatcttcagtgccaatctcattgactggtaccgccaagctccagggaagggcctggagctggtcgcagttattagtagtcgtggtatcacaagctatgcagactccgtgaagggtcgattcaccatctccagagacaacagcaagaacacgctgtatctgcaaatgaacagcctgcgggctgaggacacggccgtctattactgtcatttatttcacacagacgggttggggtattggggccaggggaccctggtcaccgtgtcttctgacatccagatgacccagagccctagctctctgtccgcctctgtgggcgacagagtgaccatcacatgttccgccagccaggatatctctaactacctgaattggtatcagcagaagccaggcaaggctcccaaggtgctgatctactttacatccagcctgcactctggagtgccatcccgcttctctggttccggaagcggaaccgactttaccctgacaatctcttccctgcaacctgaggatttcgccacatactattgccagcagtattccaccgtgccttggacatttggccagggcaccaaggtggagatcaagaggacagtggccgctccatccgtgttcatctttccccctagcgacgagcagctgaagagcggcaccgcctctgtggtgtgcctgctgaacaatttctacccccgggaggctaaggtgcagtggaaggtggataacgccctgcaatctggcaattcccaggagagcgtgaccgagcaggactctaaggattccacatatagcctgagttctaccctgacactgtccaaggctgactacgagaagcataaggtgtatgcctgcgaggtgacccatcagggcctgtccagccccgtgacaaagagctttaaccggggcgagtgt

SEQ ID NO: 39 - DNA, 1017 bp, Artificial Sequence
caggtgcagctcgtggagtctgggggaggcttggtgcagcctggggggtctctgagactctcctgtgcagcctctggtggcaccttcatcacctatgccatgggctggttccgccaagctccagggaagggcctggagtttgtcgcaggtattagttggagtggtagtagcacatactatgcagactccgtgaagggccgattcaccatctccagagacaacagcaagaacacgctgtatctgcaaatgaacagcctgcgggctgaggacacggccgtttattactgtgcagccaaaatctcgggggcgactagagagcacctaaggacttcgtatgactactggggccaggggaccctggtcaccgtgtcttctgacatccagatgacccagagccctagctctctgtccgcctctgtgggcgacagagtgaccatcacatgttccgccagccaggatatctctaactacctgaattggtatcagcagaagccaggcaaggctcccaaggtgctgatctactttacatccagcctgcactctggagtgccatcccgcttctctggttccggaagcggaaccgactttaccctgacaatctcttccctgcaacctgaggatttcgccacatactattgccagcagtattccaccgtgccttggacatttggccagggcaccaaggtggagatcaagaggacagtggccgctccatccgtgttcatctttccccctagcgacgagcagctgaagagcggcaccgcctctgtggtgtgcctgctgaacaatttctacccccgggaggctaaggtgcagtggaaggtggataacgccctgcaatctggcaattcccaggagagcgtgaccgagcaggactctaaggattccacatatagcctgagttctaccctgacactgtccaaggctgactacgagaagcataaggtgtatgcctgcgaggtgacccatcagggcctgtccagccccgtgacaaagagctttaaccggggcgagtgt

SEQ ID NO: 40 - DNA, 1014 bp, Artificial Sequence
caggtgcagctcgtggagtctgggggaggcttggtgcagcctggggggtctctgagactctcctgtgcagcctctggacgccccttcattacctatgccatgggctggttccgccaagctccagggaagggcctggagtttgtcgcagctattaactggagcggtagtatcacagcctatgcagactccgtgaagggtcgattcaccatctccagagacaacagcaagaacacgctgtatctgcaaatgaacagcctgcgggctgaggacacggccgtctattactgtgcaagtaaacgtacggcagtagctcccagagccttaaatgactatgacttctggggccaggggaccctggtcaccgtgtcttctgacatccagatgacccagagccctagctctctgtccgcctctgtgggcgacagagtgaccatcacatgttccgccagccaggatatctctaactacctgaattggtatcagcagaagccaggcaaggctcccaaggtgctgatctactttacatccagcctgcactctggagtgccatcccgcttctctggttccggaagcggaaccgactttaccctgacaatctcttccctgcaacctgaggatttcgccacatactattgccagcagtattccaccgtgccttggacatttggccagggcaccaaggtggagatcaagaggacagtggccgctccatccgtgttcatctttccccctagcgacgagcagctgaagagcggcaccgcctctgtggtgtgcctgctgaacaatttctacccccgggaggctaaggtgcagtggaaggtggataacgccctgcaatctggcaattcccaggagagcgtgaccgagcaggactctaaggattccacatatagcctgagttctaccctgacactgtccaaggctgactacgagaagcataaggtgtatgcctgcgaggtgacccatcagggcctgtccagccccgtgacaaagagctttaaccggggcgagtgt

SEQ ID NO: 41 - DNA, 1011 bp, Artificial Sequence
caggtgcagctcgtggagtctgggggaggcttggtgcagcctggggggtctctgagactctcctgtgcagcctctggacgcaccttcagtacacatagcatgggctggttccgccaggctccagggaagggcctggagtttgtagcagctattaactggaatggtgatagcacatattatgcagactccgtgaagggccgattcaccatctccagagacaacagcaagaacacgctgtatctgcaaatgaacagcctgcgggctgaggacacggccgtttattactgtgcagcccgcccgggcgccccgtcgactatagtggctatgttggactactggggccaggggaccctggtcaccgtgtcttctgacatccagatgacccagagccctagctctctgtccgcctctgtgggcgacagagtgaccatcacatgttccgccagccaggatatctctaactacctgaattggtatcagcagaagccaggcaaggctcccaaggtgctgatctactttacatccagcctgcactctggagtgccatcccgcttctctggttccggaagcggaaccgactttaccctgacaatctcttccctgcaacctgaggatttcgccacatactattgccagcagtattccaccgtgccttggacatttggccagggcaccaaggtggagatcaagaggacagtggccgctccatccgtgttcatctttccccctagcgacgagcagctgaagagcggcaccgcctctgtggtgtgcctgctgaacaatttctacccccgggaggctaaggtgcagtggaaggtggataacgccctgcaatctggcaattcccaggagagcgtgaccgagcaggactctaaggattccacatatagcctgagttctaccctgacactgtccaaggctgactacgagaagcataaggtgtatgcctgcgaggtgacccatcagggcctgtccagccccgtgacaaagagctttaaccggggcgagtgt

SEQ ID NO: 42 - DNA, 1830 bp, Artificial Sequence
gaggtgcagctggtggagtctggaggaggactggtgcagccaggaggctctctgagactgtcctgcgccgctagcggctacaccttcacaaactatggcatgaattgggtgcgccaggctccaggcaagggcctggagtgggtgggctggatcaacacctacacaggcgagcccacctatgccgctgactttaagaggaggttcaccttctccctggacacctccaagagcacagcctacctccagatgaactccctgagggccgaggacaccgccgtgtactattgcgctaagtacccccactactatggctccagccattggtatttcgacgtgtggggacagggcaccctggtgacagtgtcttccgcctctaccaagggaccttccgtgtttcctctggctccaagctctaagtctacctccggaggaacagccgctctgggatgtctggtgaaggactatttccctgagccagtgaccgtgtcctggaacagcggcgccctgacctccggagtgcacacatttcctgctgtgctccagtccagcggcctgtacagcctgtcttccgtggtgaccgtgccaagctcttccctgggcacccagacatatatctgcaacgtgaatcacaagccatccaacacaaaggtggacaagaaggtggagcccaagtcctgcgacaaaactcacacatgcccaccgtgcccagcacctgaactcctgggtggaccgtcagtcttcctcttccccccaaaacccaaggacaccctcatgatctcccggacccctgaggtcacatgcgtggtggtggacgtgagccacgaagaccctgaggtcaagttcaactggtacgtggacggcgtggaggtgcataatgccaagacaaagccgcgggaggagcagtacaatagcacgtaccgtgtggtcagcgtcctcaccgtcctgcaccaggactggctgaatggcaaggagtacaagtgcaaggtctccaacaaagccctcccagcccccatcgagaaaaccatctccaaagccaaagggcagccccgagaaccacaggtgtacaccctgcccccatcccgggaggagatgaccaagaaccaggtcagcctgacctgcctggtcaaaggcttctatcccagcgacatcgccgtggagtgggagagcaatgggcagccggagaacaactacaagaccacgcctcccgtgctggactccgacggctccttcttcctctatagcaagctcaccgtggacaagagcaggtggcagcaggggaacgtcttctcatgctccgtgatgcatgaggctctgcacaaccactacacgcagaagagcctctccctgtctccgggtgctggaggaggaggaagcggaggaggaggctctggcggcggcggctcaggcggcggcggcagcggcatccccccacacgtgcagaagtccgtgaataatgacatgatcgtgaccgataacaacggcgccgtgaagtttccccagctgtgcaagttctgcgacgtgaggttctccacctgtgacaaccagaagtcctgtatgagcaactgcagcatcacctccatctgcgagaagccccaggaggtgtgtgtggccgtgtggcggaagaacgacgagaatatcaccctggagaccgtgtgtcacgaccccaagctgccctatcacgacttcatcctggaggatgctgctagccccaagtgcatcatgaaggagaagaagaagcccggcgagaccttcttcatgtgttcctgtagcagcgacgagtgcaatgataacatcatctttagcgaggagtacaacacctccaaccccgac

SEQ ID NO: 43 - DNA, 2205 bp, Artificial Sequence
caggtgcagctcgtggagtctgggggaggcttggtgcagcctggggggtctctgagactctcctgtgcagcctctggtggcaccttcatcacctatgccatgggctggttccgccaagctccagggaagggcctggagtttgtcgcaggtattagttggagtggtagtagcacatactatgcagactccgtgaagggccgattcaccatctccagagacaacagcaagaacacgctgtatctgcaaatgaacagcctgcgggctgaggacacggccgtttattactgtgcagccaaaatctcgggggcgactagagagcacctaaggacttcgtatgactactggggccaggggaccctggtcaccgtgtcttctgaggtgcagctggtggagtctggaggaggactggtgcagccaggaggctctctgagactgtcctgcgccgctagcggctacaccttcacaaactatggcatgaattgggtgcgccaggctccaggcaagggcctggagtgggtgggctggatcaacacctacacaggcgagcccacctatgccgctgactttaagaggaggttcaccttctccctggacacctccaagagcacagcctacctccagatgaactccctgagggccgaggacaccgccgtgtactattgcgctaagtacccccactactatggctccagccattggtatttcgacgtgtggggacagggcaccctggtgacagtgtcttccgcctctaccaagggaccttccgtgtttcctctggctccaagctctaagtctacctccggaggaacagccgctctgggatgtctggtgaaggactatttccctgagccagtgaccgtgtcctggaacagcggcgccctgacctccggagtgcacacatttcctgctgtgctccagtccagcggcctgtacagcctgtcttccgtggtgaccgtgccaagctcttccctgggcacccagacatatatctgcaacgtgaatcacaagccatccaacacaaaggtggacaagaaggtggagcccaagtcctgcgacaaaactcacacatgcccaccgtgcccagcacctgaactcctgggtggaccgtcagtcttcctcttccccccaaaacccaaggacaccctcatgatctcccggacccctgaggtcacatgcgtggtggtggacgtgagccacgaagaccctgaggtcaagttcaactggtacgtggacggcgtggaggtgcataatgccaagacaaagccgcgggaggagcagtacaatagcacgtaccgtgtggtcagcgtcctcaccgtcctgcaccaggactggctgaatggcaaggagtacaagtgcaaggtctccaacaaagccctcccagcccccatcgagaaaaccatctccaaagccaaagggcagccccgagaaccacaggtgtacaccctgcccccatcccgggaggagatgaccaagaaccaggtcagcctgacctgcctggtcaaaggcttctatcccagcgacatcgccgtggagtgggagagcaatgggcagccggagaacaactacaagaccacgcctcccgtgctggactccgacggctccttcttcctctatagcaagctcaccgtggacaagagcaggtggcagcaggggaacgtcttctcatgctccgtgatgcatgaggctctgcacaaccactacacgcagaagagcctctccctgtctccgggtgctggaggaggaggaagcggaggaggaggctctggcggcggcggctcaggcggcggcggcagcggcatccccccacacgtgcagaagtccgtgaataatgacatgatcgtgaccgataacaacggcgccgtgaagtttccccagctgtgcaagttctgcgacgtgaggttctccacctgtgacaaccagaagtcctgtatgagcaactgcagcatcacctccatctgcgagaagccccaggaggtgtgtgtggccgtgtggcggaagaacgacgagaatatcaccctggagaccgtgtgtcacgaccccaagctgccctatcacgacttcatcctggaggatgctgctagccccaagtgcatcatgaaggagaagaagaagcccggcgagaccttcttcatgtgttcctgtagcagcgacgagtgcaatgataacatcatctttagcgaggagtacaacacctccaaccccgac

SEQ ID NO: 44 - DNA, 2205 bp, Artificial Sequence
caggtgcagctcgtggagtctgggggaggcttggtgcagcctggggggtctctgagactctcctgtgcagcctctggtggcaccttcatcacctatgccatgggctggttccgccaagctccagggaagggcctggagtttgtcgcaggtattagttggagtggtagtagcacatactatgcagactccgtgaagggccgattcaccatctccagagacaacagcaagaacacgctgtatctgcaaatgaacagcctgcgggctgaggacacggccgtttattactgtgcagccaaaatctcgggggcgactagagagcacctaaggacttcgtatgactactggggccaggggaccctggtcaccgtgtcttctgaggtgcagctggtggagtctggaggaggactggtgcagccaggaggctctctgagactgtcctgcgccgctagcggctacaccttcacaaactatggcatgaattgggtgcgccaggctccaggcaagggcctggagtgggtgggctggatcaacacctacacaggcgagcccacctatgccgctgactttaagaggaggttcaccttctccctggacacctccaagagcacagcctacctccagatgaactccctgagggccgaggacaccgccgtgtactattgcgctaagtacccccactactatggctccagccattggtatttcgacgtgtggggacagggcaccctggtgacagtgtcttccgcctctaccaagggaccttccgtgtttcctctggctccaagctctaagtctacctccggaggaacagccgctctgggatgtctggtgaaggactatttccctgagccagtgaccgtgtcctggaacagcggcgccctgacctccggagtgcacacatttcctgctgtgctccagtccagcggcctgtacagcctgtcttccgtggtgaccgtgccaagctcttccctgggcacccagacatatatctgcaacgtgaatcacaagccatccaacacaaaggtggacaagaaggtggagcccaagtcctgcgacaaaactcacacatgcccaccgtgcccagcacctgaactcctgggtggaccgtcagtcttcctcttccccccaaaacccaaggacaccctcatgatctcccggacccctgaggtcacatgcgtggtggtggacgtgagccacgaagaccctgaggtcaagttcaactggtacgtggacggcgtggaggtgcataatgccaagacaaagccgcgggaggagcagtacgctagcacgtaccgtgtggtcagcgtcctcaccgtcctgcaccaggactggctgaatggcaaggagtacaagtgcaaggtctccaacaaagccctcccagcccccatcgagaaaaccatctccaaagccaaagggcagccccgagaaccacaggtgtacaccctgcccccatcccgggaggagatgaccaagaaccaggtcagcctgacctgcctggtcaaaggcttctatcccagcgacatcgccgtggagtgggagagcaatgggcagccggagaacaactacaagaccacgcctcccgtgctggactccgacggctccttcttcctctatagcaagctcaccgtggacaagagcaggtggcagcaggggaacgtcttctcatgctccgtgatgcatgaggctctgcacaaccactacacgcagaagagcctctccctgtctccgggtgctggaggaggaggaagcggaggaggaggctctggcggcggcggctcaggcggcggcggcagcggcatccccccacacgtgcagaagtccgtgaataatgacatgatcgtgaccgataacaacggcgccgtgaagtttccccagctgtgcaagttctgcgacgtgaggttctccacctgtgacaaccagaagtcctgtatgagcaactgcagcatcacctccatctgcgagaagccccaggaggtgtgtgtggccgtgtggcggaagaacgacgagaatatcaccctggagaccgtgtgtcacgaccccaagctgccctatcacgacttcatcctggaggatgctgctagccccaagtgcatcatgaaggagaagaagaagcccggcgagaccttcttcatgtgttcctgtagcagcgacgagtgcaatgataacatcatctttagcgaggagtacaacacctccaaccccgac

SEQ ID NO: 45 - DNA, 2205 bp, Artificial Sequence
caggtgcagctcgtggagtctgggggaggcttggtgcagcctggggggtctctgagactctcctgtgcagcctctggtggcaccttcatcacctatgccatgggctggttccgccaagctccagggaagggcctggagtttgtcgcaggtattagttggagtggtagtagcacatactatgcagactccgtgaagggccgattcaccatctccagagacaacagcaagaacacgctgtatctgcaaatgaacagcctgcgggctgaggacacggccgtttattactgtgcagccaaaatctcgggggcgactagagagcacctaaggacttcgtatgactactggggccaggggaccctggtcaccgtgtcttctgaggtgcagctggtggagtctggaggaggactggtgcagccaggaggctctctgagactgtcctgcgccgctagcggctacaccttcacaaactatggcatgaattgggtgcgccaggctccaggcaagggcctggagtgggtgggctggatcaacacctacacaggcgagcccacctatgccgctgactttaagaggaggttcaccttctccctggacacctccaagagcacagcctacctccagatgaactccctgagggccgaggacaccgccgtgtactattgcgctaagtacccccactactatggctccagccattggtatttcgacgtgtggggacagggcaccctggtgacagtgtcttccgcctctaccaagggaccttccgtgtttcctctggctccaagctctaagtctacctccggaggaacagccgctctgggatgtctggtgaaggactatttccctgagccagtgaccgtgtcctggaacagcggcgccctgacctccggagtgcacacatttcctgctgtgctccagtccagcggcctgtacagcctgtcttccgtggtgaccgtgccaagctcttccctgggcacccagacatatatctgcaacgtgaatcacaagccatccaacacaaaggtggacaagaaggtggagcccaagtcctgcgacaaaactcacacatgcccaccgtgcccagcacctgaactcctgggtggaccgtcagtcttcctcttccccccaaaacccaaggacaccctcatgatctcccggacccctgaggtcacatgcgtggtggtggacgtgagccacgaagaccctgaggtcaagttcaactggtacgtggacggcgtggaggtgcataatgccaagacaaagccgcgggaggagcagtacaatagcacgtaccgtgtggtcagcgtcctcaccgtcctgcaccaggactggctgaatggcaaggagtacaagtgcaaggtctccaacaaagccctcccagcccccatcgagaaaaccatctccaaagccaaagggcagccccgagaaccacaggtgtacaccctgcccccatcccgggaggagatgaccaagaaccaggtcagcctgacctgcctggtcaaaggcttctatcccagcgacatcgccgtggagtgggagagcaatgggcagccggagaacaactacaagaccacgcctcccgtgctggactccgacggctccttcttcctctatagcaagctcaccgtggacaagagcaggtggcagcaggggaacgtcttctcatgctccgtgatgcatgaggctctgcacaaccactacacgcagaagagcctctccctgtctccgggtgctggaggaggaggaagcggaggaggaggctctggcggcggcggctcaggcggcggcggcagcaccatccccccacacgtgcagaagtccgtgaataatgacatgatcgtgaccgataacaacggcgccgtgaagtttccccagctgtgcaagttctgcgacgtgaggttctccacctgtgacaaccagaagtcctgtatgagcaactgcagcatcacctccatctgcgagaagccccaggaggtgtgtgtggccgtgtggcggaagaacgacgagaatatcaccctggagaccgtgtgtcacgaccccaagctgccctatcacgacttcatcctggaggatgctgctagccccaagtgcatcatgaaggagaagaagaagcccggcgagaccttcttcatgtgttcctgtagcagcgacgagtgcaatgataacatcatctttagcgaggagtacaacacctccaaccccgac

SEQ ID NO: 46 - DNA, 642 bp, Artificial Sequence
gacatccagatgacccagagccctagctctctgtccgcctctgtgggcgacagagtgaccatcacatgttccgccagccaggatatctctaactacctgaattggtatcagcagaagccaggcaaggctcccaaggtgctgatctactttacatccagcctgcactctggagtgccatcccgcttctctggttccggaagcggaaccgactttaccctgacaatctcttccctgcaacctgaggatttcgccacatactattgccagcagtattccaccgtgccttggacatttggccagggcaccaaggtggagatcaagaggacagtggccgctccatccgtgttcatctttccccctagcgacgagcagctgaagagcggcaccgcctctgtggtgtgcctgctgaacaatttctacccccgggaggctaaggtgcagtggaaggtggataacgccctgcaatctggcaattcccaggagagcgtgaccgagcaggactctaaggattccacatatagcctgagttctaccctgacactgtccaaggctgactacgagaagcataaggtgtatgcctgcgaggtgacccatcagggcctgtccagccccgtgacaaagagctttaaccggggcgagtgt

SEQ ID NO: 47 - protein, 356 aa, Artificial Sequence
QVQLVESGGGLVQPGGSLRLSCAASGGTFITYAMGWFRQAPGKGLEFVAGISWSGSSTYYADSVKGRFTISRDNSKNTLYLQMNSLRAEDTAVYYCAAKISGATREHLRTSYDYWGQGTLVTVSSEPKSCDKTHTCPPCPAPELLGGPSVFLFPPKPKDTLMISRTPEVTCVVVDVSHEDPEVKFNWYVDGVEVHNAKTKPREEQYNSTYRVVSVLTVLHQDWLNGKEYKCKVSNKALPAPIEKTISKAKGQPREPQVYTLPPSRDELTKNQVSLTCLVKGFYPSDIAVEWESNGQPENNYKTTPPVLDSDGSFFLYSKLTVDKSRWQQGNVFSCSVMHEALHNHYTQKSLSLSPG

SEQ ID NO: 48 - protein, 389 aa, Artificial Sequence
EPKSCDKTHTCPPCPAPELLGGPSVFLFPPKPKDTLMISRTPEVTCVVVDVSHEDPEVKFNWYVDGVEVHNAKTKPREEQYASTYRVVSVLTVLHQDWLNGKEYKCKVSNKALPAPIEKTISKAKGQPREPQVYTLPPSREEMTKNQVSLTCLVKGFYPSDIAVEWESNGQPENNYKTTPPVLDSDGSFFLYSKLTVDKSRWQQGNVFSCSVMHEALHNHYTQKSLSLSPGAGGGGSGGGGSGGGGSGGGGSGIPPHVQKSVNNDMIVTDNNGAVKFPQLCKFCDVRFSTCDNQKSCMSNCSITSICEKPQEVCVAVWRKNDENITLETVCHDPKLPYHDFILEDAASPKCIMKEKKKPGETFFMCSCSSDECNDNIIFSEEYNTSNPD

SEQ ID NO: 49 - protein, 25 aa, Artificial Sequence
QVQLVESGGGLVQPGGSLRLSCAAS

SEQ ID NO: 50 - protein, 17 aa, Artificial Sequence
IDWYRQAPGKGLELVAV

SEQ ID NO: 51 - protein, 17 aa, Artificial Sequence
MGWFRQAPGKGLEFVAG

SEQ ID NO: 52 - protein, 17 aa, Artificial Sequence
MGWFRQAPGKGLEFVAA

SEQ ID NO: 53 - protein, 38 aa, Artificial Sequence
SYADSVKGRFTISRDNSKNTLYLQMNSLRAEDTAVYYC

SEQ ID NO: 54 - protein, 38 aa, Artificial Sequence
YYADSVKGRFTISRDNSKNTLYLQMNSLRAEDTAVYYC

SEQ ID NO: 55 - protein, 38 aa, Artificial Sequence
AYADSVKGRFTISRDNSKNTLYLQMNSLRAEDTAVYYC

SEQ ID NO: 56 - protein, 11 aa, Artificial Sequence
WGQGTLVTVSS